European Patent Specification EP 3 129 404 B1, published January 28, 2026. Title: Immunoglobulins binding human Vgamma9 Vdelta2 T cell receptors. Applicant: Stichting VU-VUmc. The sequence listing filed with the application follows.

SEQUENCE LISTING (72 sequences)

SEQ ID NO: 1 - protein, 10 aa, Llama glama
GRTFSRYTMG

SEQ ID NO: 2 - protein, 17 aa, Llama glama
AISWSGGRTNFAGSVKG

SEQ ID NO: 3 - protein, 13 aa, Llama glama
DWLPVPGRESYDY

SEQ ID NO: 4 - protein, 10 aa, Llama glama
GRTFSSYAMG

SEQ ID NO: 5 - protein, 17 aa, Llama glama
AISWSGGTTYYADSVKG

SEQ ID NO: 6 - protein, 16 aa, Llama glama
SLDCSGPGCHTAEYDY

SEQ ID NO: 7 - protein, 10 aa, Llama glama
GRTFSEYAMG

SEQ ID NO: 8 - protein, 17 aa, Llama glama
AISWTGSKTYYADSVKG

SEQ ID NO: 9 - protein, 16 aa, Llama glama
SSDCSGPGCHTEEYDY

SEQ ID NO: 10 - protein, 17 aa, Llama glama
AVSWSGGSTYYADSVKG

SEQ ID NO: 11 - protein, 16 aa, Llama glama
SQDCSGPGCYTNEYDS

SEQ ID NO: 12 - protein, 10 aa, Llama glama
GSIFSNYAMA

SEQ ID NO: 13 - protein, 17 aa, Llama glama
AVSWSGGRTYYADSVKG

SEQ ID NO: 14 - protein, 16 aa, Llama glama
SLSCSGPGCSLEEYDY

SEQ ID NO: 15 - protein, 10 aa, Llama glama
GRPFSNYAMG

SEQ ID NO: 16 - protein, 17 aa, Llama glama
VISWSGGSTYYADSVKG

SEQ ID NO: 17 - protein, 18 aa, Llama glama
QFSGASTVVAGTALDYDY

SEQ ID NO: 18 - protein, 10 aa, Llama glama
GRPFSNYGMG

SEQ ID NO: 19 - protein, 17 aa, Llama glama
GISWSGGSTDYADSVKG

SEQ ID NO: 20 - protein, 17 aa, Llama glama
VFSGAETAYYPSDDYDY

SEQ ID NO: 21 - protein, 17 aa, Llama glama
GITWSGGSTHYADLVKG

SEQ ID NO: 22 - protein, 17 aa, Llama glama
VFSGAETAYYPSTEYDY

SEQ ID NO: 23 - protein, 10 aa, Llama glama
GRPFNNYGMG

SEQ ID NO: 24 - protein, 17 aa, Llama glama
GISWSGGSTYYADSVKG

SEQ ID NO: 25 - protein, 17 aa, Llama glama
VFSGAETAQYPSYDYDY

SEQ ID NO: 26 - protein, 17 aa, Llama glama
AVTWSGGSTYYADSVKG

SEQ ID NO: 27 - protein, 20 aa, Llama glama
QFNGAENIVPATTTPTSYDY

SEQ ID NO: 28 - protein, 17 aa, Llama glama
AISWSGGSTSYADSVKG

SEQ ID NO: 29 - protein, 21 aa, Llama glama
QFSGADYGFGRLGIRGYEYDY

SEQ ID NO: 30 - protein, 21 aa, Llama glama
QFSGADYGFGRLGIQGYEYDY

SEQ ID NO: 31 - protein, 10 aa, Llama glama
GRTFSNYAMG

SEQ ID NO: 32 - protein, 17 aa, Llama glama
AISWSGGSTYYADSVKG

SEQ ID NO: 33 - protein, 21 aa, Llama glama
MFSGSESQLVVVITNLYEYDY

SEQ ID NO: 34 - protein, 17 aa, Llama glama
TISWSGGSTYYADSVKG

SEQ ID NO: 35 - protein, 18 aa, Llama glama
AFSGSDYANTKKEVEYDY

SEQ ID NO: 36 - protein, 17 aa, Llama glama
AISWSGGMTDHADSVKG

SEQ ID NO: 37 - protein, 21 aa, Llama glama
AFAGDIPYGSSWYGDPTTYDY

SEQ ID NO: 38 - protein, 10 aa, Llama glama
GRTSSTFSMA

SEQ ID NO: 39 - protein, 17 aa, Llama glama
AINWSGGSTRYADSVSD

SEQ ID NO: 40 - protein, 15 aa, Llama glama
RRGGIYYSTQNDYDY

SEQ ID NO: 41 - protein, 10 aa, Llama glama
VRTFSDYRMG

SEQ ID NO: 42 - protein, 17 aa, Llama glama
TISWSGGLTYYADSVKG

SEQ ID NO: 43 - protein, 14 aa, Llama glama
GGGYAGGTYYHPEE

SEQ ID NO: 44 - protein, 10 aa, Llama glama
GFTFDDYCIA

SEQ ID NO: 45 - protein, 17 aa, Llama glama
CITTSDGSTYYADSVKG

SEQ ID NO: 46 - protein, 18 aa, Llama glama
YFGYGCYGGAQDYRAMDY

SEQ ID NO: 47 - protein, 122 aa, Llama glama
EVQLVESGGGLVQAGDSLRLSCAASGRTFSRYTMGWFRQAPGKEREFVAAISWSGGRTNFAGSVKGRFTISRDNAKNTVYLQMNSLKPEDTAVYYCAADWLPVPGRESYDYWGQGTQVTVSS

SEQ ID NO: 48 - protein, 125 aa, Llama glama
EVQLVESGGGLVQAGGSLRLSCTASGRTFSSYAMGWFRQAPGKEREFVAAISWSGGTTYYADSVKGRFTISRDNAKNTVSLQMNSLKPEDTAVYFCAASLDCSGPGCHTAEYDYWGQGTQVTVSS

SEQ ID NO: 49 - protein, 125 aa, Llama glama
EVQLVESGGGLVQAGGSLRLSCAATGRTFSEYAMGWFRQAPGKEREFAAAISWTGSKTYYADSVKGRFTISRDNAKNTVYLQMNSLKPEDTAVYYCAASSDCSGPGCHTEEYDYWGQGTQVTVSS

SEQ ID NO: 50 - protein, 125 aa, Llama glama
EVQLVESGGGLVQAGGSLRLSCAASGRTFSSYAMGWFRQAPGKEREFVAAVSWSGGSTYYADSVKGRFTISRDNARNTVYLQMNSLNPEDTAVYYCAASQDCSGPGCYTNEYDSWGQGTQVTVSS

SEQ ID NO: 51 - protein, 125 aa, Llama glama
EVQLVESGGGLVQPGGSLRLSCAASGSIFSNYAMAWFRQAPEKERDFLAAVSWSGGRTYYADSVKGRFTISRDNAKNTVNLQMNSLKPEDTAVYYCAASLSCSGPGCSLEEYDYWGQGTQVTVSS

SEQ ID NO: 52 - protein, 127 aa, Llama glama
EVQLVESGGGLVQAGGSLRLSCAASGRPFSNYAMGWFRQAPGKEREFVTVISWSGGSTYYADSVKGRFTISRDNAKNTVYLQMNSLKPEDTAVYYCAAQFSGASTVVAGTALDYDYWGQGTRVTVSS

SEQ ID NO: 53 - protein, 126 aa, Llama glama
EVQLVESGGGLVQAGGSLRLSCAASGRPFSNYGMGWFRQAPGKKREFVAGISWSGGSTDYADSVKGRLTISRDNAKNTVYLQMNSLKPEDTAVYYCAAVFSGAETAYYPSDDYDYWGQGTQVTVSS

SEQ ID NO: 54 - protein, 126 aa, Llama glama
EVQLVESGGGLVQAGGSLRLSCAASGRPFSNYGMGWFRQAPGKKREFVAGISWSGGSTDYADSVKGRFTISRDNAKNTVYLQMNSLKPEDTAVYYCAAVFSGAETAYYPSDDYDYWGQGTQVTVSS

SEQ ID NO: 55 - protein, 126 aa, Llama glama
EVQLVESGGGLVQAGGSLRLSCAASGRPFSNYGMGWFRQAPGKKRESVAGISWSGGSTDYADSVKGRFTISRDNAKNTVYLQMNSLKPEDTAVYYCAAVFSGAETAYYPSDDYDYWGQGTQVTVSS

SEQ ID NO: 56 - protein, 126 aa, Llama glama
EVQLVESGGGLVQAGGSLRLSCAVSGRPFSNYGMGWFRQAPGKEREFVAGITWSGGSTHYADLVKGRFTISRDNAKNTVHLQMNSLKPEDTAVYYCAAVFSGAETAYYPSTEYDYWGQGTQVTVSS

SEQ ID NO: 57 - protein, 126 aa, Llama glama
EVQLVESGGGLVQAGGSLRLSCAASGRPFNNYGMGWFRQAPGKEREFVAGISWSGGSTYYADSVKGRFTISRDNAKNTVYLQMNSLKPEDTAVYYCAAVFSGAETAQYPSYDYDYWGQGTQVTVSS

SEQ ID NO: 58 - protein, 129 aa, Llama glama
EVQLVESGGGLVQAGGSLRLSCVASGRPFSNYAMGWFRQAPGKEREFVAAVTWSGGSTYYADSVKGRFAISRDNAKNTVYLQMNSLKPEDTAVYYCAAQFNGAENIVPATTTPTSYDYWGQGTQVTVSS

SEQ ID NO: 59 - protein, 130 aa, Llama glama
EVQLVESGGGLVQAGGSLRLSCAASGRPFSNYAMGWFRQAPGKEREFVAAISWSGGSTSYADSVKGRFTISRDNAKNTVYLQMNSPKPEDTAIYYCAAQFSGADYGFGRLGIRGYEYDYWGQGTQVTVSS

SEQ ID NO: 60 - protein, 130 aa, Llama glama
EVQLVESGGGLVQAGGSLRLSCAASGRPFSNYAMGWFRQAPGKEREFVAAISWSGGSTSYADSVKGRFTISRDNAENTVYLQMNSPKPEDTAIYYCAAQFSGADYGFGRLGIQGYEYDYWGQGTQVTVSS

SEQ ID NO: 61 - protein, 130 aa, Llama glama
EVQLVESGGGLVQAGGSLRLSCAASGRTFSNYAMGWFRQAPGKEREFVAAISWSGGSTYYADSVKGRFTISRDNAKNTVYLQMNSLKPEDTAVYYCAAMFSGSESQLVVVITNLYEYDYWGQGTQVTVSS

SEQ ID NO: 62 - protein, 127 aa, Llama glama
EVQLVESGGGLVQAGGSLRLSCAASGRTFSNYAMGWFRQAPGKEREFVATISWSGGSTYYADSVKGRFTISRDNAKNTVYLQMNSLKPEDTAVYYCAAAFSGSDYANTKKEVEYDYWGQGTQVTVSS

SEQ ID NO: 63 - protein, 130 aa, Llama glama
EVQLVESGGGLVQAGGSLRLSCIASGRTFSNYAMGWFRQAPGKEREFVAAISWSGGMTDHADSVKGRFTISRDNAKNTVYLQMNSLKPEDTAVYYCAAAFAGDIPYGSSWYGDPTTYDYWGQGTQVTVSS

SEQ ID NO: 64 - protein, 124 aa, Llama glama
EVQLVESGGGLVQAGGSLRLSCAASGRTSSTFSMAWFRQAPRKEREFVAAINWSGGSTRYADSVSDRFAISRDNAKNTVYLQMNNLKPEDTAVYYCAARRGGIYYSTQNDYDYWGQGTQVTVSS

SEQ ID NO: 65 - protein, 123 aa, Llama glama
EVQLVESGGGLVQAGGSLRLSCAVSVRTFSDYRMGWFRQAPGKEREFVSTISWSGGLTYYADSVKGRFTISRDNSKNTLYLQMNSLKPEDTAVYYCAAGGGYAGGTYYHPEEWGQGTQVTVSS

SEQ ID NO: 66 - protein, 127 aa, Llama glama
EVQLVESGGGLVQAGGSLRLSCAASGFTFDDYCIAWFRQAPGKEREPVSCITTSDGSTYYADSVKGRFTISSDNAKNTVYLQMNRLKPEDTAVYYCAAYFGYGCYGGAQDYRAMDYWGKGTLVTVSS

SEQ ID NO: 67 - protein, 25 aa, Llama glama
EVQLVESGGGLVQAGDSLRLSCAAS

SEQ ID NO: 68 - protein, 14 aa, Llama glama
WFRQAPGKEREFVA

SEQ ID NO: 69 - protein, 32 aa, Llama glama
RFTISRDNAKNTVYLQMNSLKPEDTAVYYCAA

SEQ ID NO: 70 - protein, 11 aa, Llama glama
WGQGTQVTVSS

SEQ ID NO: 71 - protein, 315 aa, Homo Sapiens
MLSLLHASTLAVLGALCVYGAGHLEQPQISSTKTLSKTARLECVVSGITISATSVYWYRERPGEVIQFLVSISYDGTVRKESGIPSGKFEVDRIPETSTSTLTIHNVEKQDIATYYCALWEAQQELGKKIKVFGPGTKLIITDKQLDADVSPKPTIFLPSIAETKLQKAGTYLCLLEKFFPDVIKIHWEEKKSNTILGSQEGNTMKTNDTYMKFSWLTVPEKSLDKEHRCIVRHENNKNGVDQEIIFPPIKTDVITMDPKDNCSKDANDTLLLQLTNTSAYYMYLLLLLKSVVYFAIITCCLLRRTAFCCNGEKS

SEQ ID NO: 72 - protein, 292 aa, Homo Sapiens [sequence omitted]